European Patent Specification EP 3 966 573 B1, published April 22, 2026. Title: Novel Ligand Assays. Applicant: Otago Innovation Limited. The sequence listing filed with the application follows.

SEQUENCE LISTING (80 sequences)

SEQ ID NO: 1 - DNA, 18 bp, Artificial
  T7 RNA polymerase promoter/initiator sequence
taatacgactcactatag

SEQ ID NO: 2 - DNA, 18 bp, Artificial
  T3 RNA polymerase promoter/initiator sequence
aattaaccctcactaaag

SEQ ID NO: 3 - DNA, 18 bp, Artificial
  SP6 RNA polymerase promoter/initiator sequence
atttaggtgacactatag

SEQ ID NO: 4 - DNA, 15 bp, Artificial
  Androgen Response Element 1 - Sense Strand
  misc_feature (7)..(9): n is a, c, g, or t
agaacannntgttct

SEQ ID NO: 5 - DNA, 15 bp, Artificial
  Androgen Response Element 1 - Antisense Strand
  misc_feature (7)..(9): n is a, c, g, or t
tcttgtnnnacaaga

SEQ ID NO: 6 - DNA, 15 bp, Artificial
  Androgen Response Element 2 - Sense Strand
  misc_feature (7)..(9): n is a, c, g, or t
ggtacannntgttct

SEQ ID NO: 7 - DNA, 15 bp, Artificial
  Androgen Response Element 2 - Antisense Strand
  misc_feature (7)..(9): n is a, c, g, or t
ccatgtnnnacaaga

SEQ ID NO: 8 - DNA, 15 bp, Artificial
  Estrogen Response Element - Sense Strand
  misc_feature (7)..(9): n is a, c, g, or t
aggtcannntgacct

SEQ ID NO: 9 - DNA, 15 bp, Artificial
  Estrogen Response Element - Sense Strand
  misc_feature (7)..(9): n is a, c, g, or t
tccagtnnnactgga

SEQ ID NO: 10 - DNA, 15 bp, Artificial
  Progesterone Response Element - Sense Strand
ggtacaaactgttct

SEQ ID NO: 11 - DNA, 15 bp, Artificial
  Progesterone Response Element - Antisense Strand
ccatgtttgacaaga

SEQ ID NO: 12 - DNA, 15 bp, Artificial
  Glucocorticoid/Mineralocorticoid Response Element - Sense Strand
  misc_feature (7)..(7): n is a, c, g, or t
agaacanaatgttct

SEQ ID NO: 13 - DNA, 15 bp, Artificial
  Glucocorticoid/Mineralocorticoid Response Element - Antisense Strand
  misc_feature (7)..(7): n is a, c, g, or t
tcttgtnttacaaga

SEQ ID NO: 14 - DNA, 146 bp, Artificial
  T7i-ARE-F30MangoII
taatacgactcactatagactctggaggaatggagaacagcctgttctccattgccatgtgtatgtgggtacgaaggagaggagaggaagaggagagtacccacatactctgatgatccttcgggatcattcatggcaatctagga

SEQ ID NO: 15 - DNA, 142 bp, Artificial
  T7i-ERE-F30MangoII
taatacgactcactatagactctggaggaacaggtcagcatgacctgttgccatgtgtatgtgggtacgaaggagaggagaggaagaggagagtacccacatactctgatgatccttcgggatcattcatggcaatctagga

SEQ ID NO: 16 - DNA, 140 bp, Artificial
  T7i-PRE-F30MangoII
taatacgactcactatagactctggaggaaggtacaaactgttctttgccatgtgtatgtgggtacgaaggagaggagaggaagaggagagtacccacatactctgatgatccttcgggatcattcatggcaatctagga

SEQ ID NO: 17 - DNA, 140 bp, Artificial
  T7i-MRE-F30MangoII
taatacgactcactatagactctggaggaatgtacaggatgttctttgccatgtgtatgtgggtacgaaggagaggagaggaagaggagagtacccacatactctgatgatccttcgggatcattcatggcaatctagga

SEQ ID NO: 18 - DNA, 140 bp, Artificial; identical to SEQ ID NO: 17
  T7i-GRE-F30MangoII

SEQ ID NO: 19 - DNA, 81 bp, Artificial
  T7i-ARE-MangoII
taatacgactcactatagactctggaggaatggagaacagcctgttctccatacgaaggagaggagaggaagaggagagta

SEQ ID NO: 20 - DNA, 77 bp, Artificial
  T7i-ERE-MangoII
taatacgactcactatagactctggaggaacaggtcagcatgacctgtacgaaggagaggagaggaagaggagagta

SEQ ID NO: 21 - DNA, 75 bp, Artificial
  T7i-PRE-MangoII
taatacgactcactatagactctggaggaaggtacaaactgttcttacgaaggagaggagaggaagaggagagta

SEQ ID NO: 22 - DNA, 75 bp, Artificial
  T7i-MRE-MangoII
taatacgactcactatagactctggaggaatgtacaggatgttcttacgaaggagaggagaggaagaggagagta

SEQ ID NO: 23 - DNA, 75 bp, Artificial; identical to SEQ ID NO: 22
  T7i-GRE-MangoII

SEQ ID NO: 24 - DNA, 120 bp, Artificial
  T7i-ARE-iSpinach
taatacgactcactatagactctggaggaatggagaacagcctgttctccaaggagtacggtgagggtcgggtccagtaggtacgcctactgttgagtagagtgtgggctccgtactccc

SEQ ID NO: 25 - DNA, 116 bp, Artificial
  T7i-ERE-iSpinach
taatacgactcactatagactctggaggaacaggtcagcatgacctgaggagtacggtgagggtcgggtccagtaggtacgcctactgttgagtagagtgtgggctccgtactccc

SEQ ID NO: 26 - DNA, 114 bp, Artificial
  T7i-PRE-iSpinach
taatacgactcactatagactctggaggaaggtacaaactgttctaggagtacggtgagggtcgggtccagtaggtacgcctactgttgagtagagtgtgggctccgtactccc

SEQ ID NO: 27 - DNA, 114 bp, Artificial
  T7i-MRE-iSpinach
taatacgactcactatagactctggaggaatgtacaggatgttctaggagtacggtgagggtcgggtccagtaggtacgcctactgttgagtagagtgtgggctccgtactccc

SEQ ID NO: 28 - DNA, 114 bp, Artificial; identical to SEQ ID NO: 27
  T7i-GRE-iSpinach

SEQ ID NO: 29 - DNA, 190 bp, Artificial
  T7i-ARE-F30iSpinach
taatacgactcactatagactctggaggaatggagaacagcctgttctccattgccatgtgtatgtgggaggagtacggtgagggtcgggtccagtaggtacgcctactgttgagtagagtgtgggctccgtactccccccacatactctgatgatccttcgggatcattcatggcaatctagatctaga

SEQ ID NO: 30 - DNA, 186 bp, Artificial
  T7i-ERE-F30iSpinach
taatacgactcactatagactctggaggaacaggtcagcatgacctgttgccatgtgtatgtgggaggagtacggtgagggtcgggtccagtaggtacgcctactgttgagtagagtgtgggctccgtactccccccacatactctgatgatccttcgggatcattcatggcaatctagatctaga

SEQ ID NO: 31 - DNA, 184 bp, Artificial
  T7i-PRE-F30iSpinach
taatacgactcactatagactctggaggaaggtacaaactgttctttgccatgtgtatgtgggaggagtacggtgagggtcgggtccagtaggtacgcctactgttgagtagagtgtgggctccgtactccccccacatactctgatgatccttcgggatcattcatggcaatctagatctaga

SEQ ID NO: 32 - DNA, 184 bp, Artificial
  T7i-MRE-F30iSpinach
taatacgactcactatagactctggaggaatgtacaggatgttctttgccatgtgtatgtgggaggagtacggtgagggtcgggtccagtaggtacgcctactgttgagtagagtgtgggctccgtactccccccacatactctgatgatccttcgggatcattcatggcaatctagatctaga

SEQ ID NO: 33 - DNA, 184 bp, Artificial; identical to SEQ ID NO: 32
  T7i-GRE-F30iSpinach

SEQ ID NO: 34 - DNA, 81 bp, Artificial
  T3i-ARE-MangoII
aattaaccctcactaaagactctggaggaatggagaacagcctgttctccatacgaaggagaggagaggaagaggagagta

SEQ ID NO: 35 - DNA, 77 bp, Artificial
  T3i-ERE-MangoII
aattaaccctcactaaagactctggaggaacaggtcagcatgacctgtacgaaggagaggagaggaagaggagagta

SEQ ID NO: 36 - DNA, 75 bp, Artificial
  T3i-PRE-MangoII
aattaaccctcactaaagactctggaggaaggtacaaactgttcttacgaaggagaggagaggaagaggagagta

SEQ ID NO: 37 - DNA, 75 bp, Artificial
  T3i-MRE-MangoII
aattaaccctcactaaagactctggaggaatgtacaggatgttcttacgaaggagaggagaggaagaggagagta

SEQ ID NO: 38 - DNA, 75 bp, Artificial; identical to SEQ ID NO: 37
  T3i-GRE-MangoII

SEQ ID NO: 39 - DNA, 146 bp, Artificial
  T3i-ARE-F30MangoII
aattaaccctcactaaagactctggaggaatggagaacagcctgttctccattgccatgtgtatgtgggtacgaaggagaggagaggaagaggagagtacccacatactctgatgatccttcgggatcattcatggcaatctagga

SEQ ID NO: 40 - DNA, 142 bp, Artificial
  T3i-ERE-F30MangoII
aattaaccctcactaaagactctggaggaacaggtcagcatgacctgttgccatgtgtatgtgggtacgaaggagaggagaggaagaggagagtacccacatactctgatgatccttcgggatcattcatggcaatctagga

SEQ ID NO: 41 - DNA, 140 bp, Artificial
  T3i-PRE-F30MangoII
aattaaccctcactaaagactctggaggaaggtacaaactgttctttgccatgtgtatgtgggtacgaaggagaggagaggaagaggagagtacccacatactctgatgatccttcgggatcattcatggcaatctagga

SEQ ID NO: 42 - DNA, 140 bp, Artificial
  T3i-MRE-F30MangoII
aattaaccctcactaaagactctggaggaatgtacaggatgttctttgccatgtgtatgtgggtacgaaggagaggagaggaagaggagagtacccacatactctgatgatccttcgggatcattcatggcaatctagga

SEQ ID NO: 43 - DNA, 140 bp, Artificial; identical to SEQ ID NO: 42
  T3i-GRE-F30MangoII

SEQ ID NO: 44 - DNA, 120 bp, Artificial
  T3i-ARE-iSpinach
aattaaccctcactaaagactctggaggaatggagaacagcctgttctccaaggagtacggtgagggtcgggtccagtaggtacgcctactgttgagtagagtgtgggctccgtactccc

SEQ ID NO: 45 - DNA, 116 bp, Artificial
  T3i-ERE-iSpinach
aattaaccctcactaaagactctggaggaacaggtcagcatgacctgaggagtacggtgagggtcgggtccagtaggtacgcctactgttgagtagagtgtgggctccgtactccc

SEQ ID NO: 46 - DNA, 114 bp, Artificial
  T3i-PRE-iSpinach
aattaaccctcactaaagactctggaggaaggtacaaactgttctaggagtacggtgagggtcgggtccagtaggtacgcctactgttgagtagagtgtgggctccgtactccc

SEQ ID NO: 47 - DNA, 114 bp, Artificial
  T3i-MRE-iSpinach
aattaaccctcactaaagactctggaggaatgtacaggatgttctaggagtacggtgagggtcgggtccagtaggtacgcctactgttgagtagagtgtgggctccgtactccc

SEQ ID NO: 48 - DNA, 114 bp, Artificial; identical to SEQ ID NO: 47
  T3i-GRE-iSpinach

SEQ ID NO: 49 - DNA, 190 bp, Artificial
  T3i-ARE-F30iSpinach
aattaaccctcactaaagactctggaggaatggagaacagcctgttctccattgccatgtgtatgtgggaggagtacggtgagggtcgggtccagtaggtacgcctactgttgagtagagtgtgggctccgtactccccccacatactctgatgatccttcgggatcattcatggcaatctagatctaga

SEQ ID NO: 50 - DNA, 186 bp, Artificial
  T3i-ERE- F30iSpinach
aattaaccctcactaaagactctggaggaacaggtcagcatgacctgttgccatgtgtatgtgggaggagtacggtgagggtcgggtccagtaggtacgcctactgttgagtagagtgtgggctccgtactccccccacatactctgatgatccttcgggatcattcatggcaatctagatctaga

SEQ ID NO: 51 - DNA, 184 bp, Artificial
  T3i-PRE- F30iSpinach
aattaaccctcactaaagactctggaggaaggtacaaactgttctttgccatgtgtatgtgggaggagtacggtgagggtcgggtccagtaggtacgcctactgttgagtagagtgtgggctccgtactccccccacatactctgatgatccttcgggatcattcatggcaatctagatctaga

SEQ ID NO: 52 - DNA, 184 bp, Artificial
  T3i-MRE- F30iSpinach
aattaaccctcactaaagactctggaggaatgtacaggatgttctttgccatgtgtatgtgggaggagtacggtgagggtcgggtccagtaggtacgcctactgttgagtagagtgtgggctccgtactccccccacatactctgatgatccttcgggatcattcatggcaatctagatctaga

SEQ ID NO: 53 - DNA, 184 bp, Artificial; identical to SEQ ID NO: 52
  T3i-GRE- F30iSpinach

SEQ ID NO: 54 - DNA, 81 bp, Artificial
  SP6i-ARE-MangoII
atttaggtgacactatagactctggaggaatggagaacagcctgttctccatacgaaggagaggagaggaagaggagagta

SEQ ID NO: 55 - DNA, 77 bp, Artificial
  SP6i-ERE-MangoII
atttaggtgacactatagactctggaggaacaggtcagcatgacctgtacgaaggagaggagaggaagaggagagta

SEQ ID NO: 56 - DNA, 75 bp, Artificial
  SP6i-PRE-MangoII
atttaggtgacactatagactctggaggaaggtacaaactgttcttacgaaggagaggagaggaagaggagagta

SEQ ID NO: 57 - DNA, 75 bp, Artificial
  SP6i-MRE-MangoII
atttaggtgacactatagactctggaggaatgtacaggatgttcttacgaaggagaggagaggaagaggagagta

SEQ ID NO: 58 - DNA, 75 bp, Artificial; identical to SEQ ID NO: 57
  SP6i-GRE-MangoII

SEQ ID NO: 59 - DNA, 146 bp, Artificial
  SP6i-ARE-F30MangoII
atttaggtgacactatagactctggaggaatggagaacagcctgttctccattgccatgtgtatgtgggtacgaaggagaggagaggaagaggagagtacccacatactctgatgatccttcgggatcattcatggcaatctagga

SEQ ID NO: 60 - DNA, 142 bp, Artificial
  SP6i-ERE-F30MangoII
atttaggtgacactatagactctggaggaacaggtcagcatgacctgttgccatgtgtatgtgggtacgaaggagaggagaggaagaggagagtacccacatactctgatgatccttcgggatcattcatggcaatctagga

SEQ ID NO: 61 - DNA, 140 bp, Artificial
  SP6i-PRE-F30MangoII
atttaggtgacactatagactctggaggaaggtacaaactgttctttgccatgtgtatgtgggtacgaaggagaggagaggaagaggagagtacccacatactctgatgatccttcgggatcattcatggcaatctagga

SEQ ID NO: 62 - DNA, 140 bp, Artificial
  SP6i-MRE-F30MangoII
atttaggtgacactatagactctggaggaatgtacaggatgttctttgccatgtgtatgtgggtacgaaggagaggagaggaagaggagagtacccacatactctgatgatccttcgggatcattcatggcaatctagga

SEQ ID NO: 63 - DNA, 140 bp, Artificial; identical to SEQ ID NO: 62
  SP6i-GRE-F30MangoII

SEQ ID NO: 64 - DNA, 120 bp, Artificial
  SP6i-ARE-iSpinach
atttaggtgacactatagactctggaggaatggagaacagcctgttctccaaggagtacggtgagggtcgggtccagtaggtacgcctactgttgagtagagtgtgggctccgtactccc

SEQ ID NO: 65 - DNA, 116 bp, Artificial
  SP6i-ERE-iSpinach
atttaggtgacactatagactctggaggaacaggtcagcatgacctgaggagtacggtgagggtcgggtccagtaggtacgcctactgttgagtagagtgtgggctccgtactccc

SEQ ID NO: 66 - DNA, 114 bp, Artificial
  SP6i-PRE-iSpinach
atttaggtgacactatagactctggaggaaggtacaaactgttctaggagtacggtgagggtcgggtccagtaggtacgcctactgttgagtagagtgtgggctccgtactccc

SEQ ID NO: 67 - DNA, 114 bp, Artificial
  SP6i-MRE-iSpinach
atttaggtgacactatagactctggaggaatgtacaggatgttctaggagtacggtgagggtcgggtccagtaggtacgcctactgttgagtagagtgtgggctccgtactccc

SEQ ID NO: 68 - DNA, 114 bp, Artificial; identical to SEQ ID NO: 67
  SP6i-GRE-iSpinach

SEQ ID NO: 69 - DNA, 190 bp, Artificial
  SP6i-ARE-F30iSpinach
atttaggtgacactatagactctggaggaatggagaacagcctgttctccattgccatgtgtatgtgggaggagtacggtgagggtcgggtccagtaggtacgcctactgttgagtagagtgtgggctccgtactccccccacatactctgatgatccttcgggatcattcatggcaatctagatctaga

SEQ ID NO: 70 - DNA, 186 bp, Artificial
  SP6i-ERE- F30iSpinach
atttaggtgacactatagactctggaggaacaggtcagcatgacctgttgccatgtgtatgtgggaggagtacggtgagggtcgggtccagtaggtacgcctactgttgagtagagtgtgggctccgtactccccccacatactctgatgatccttcgggatcattcatggcaatctagatctaga

SEQ ID NO: 71 - DNA, 184 bp, Artificial
  SP6i-PRE- F30iSpinach
atttaggtgacactatagactctggaggaaggtacaaactgttctttgccatgtgtatgtgggaggagtacggtgagggtcgggtccagtaggtacgcctactgttgagtagagtgtgggctccgtactccccccacatactctgatgatccttcgggatcattcatggcaatctagatctaga

SEQ ID NO: 72 - DNA, 184 bp, Artificial
  SP6i-MRE-F30iSpinach
atttaggtgacactatagactctggaggaatgtacaggatgttctttgccatgtgtatgtgggaggagtacggtgagggtcgggtccagtaggtacgcctactgttgagtagagtgtgggctccgtactccccccacatactctgatgatccttcgggatcattcatggcaatctagatctaga

SEQ ID NO: 73 - DNA, 184 bp, Artificial; identical to SEQ ID NO: 72
  SP6i-GRE-F30iSpinach

SEQ ID NO: 74 - DNA, 12 bp, Artificial
  Filler Sequence
actctggaggaa

SEQ ID NO: 75 - DNA, 67 bp, Artificial
  3xTandem Androgen Response Element
aagcttagaacagtttgtaacgagctcgttacaaactgttctagctcgttacaaactgttctaagct

SEQ ID NO: 76 - DNA, 21 bp, Artificial
  Primary Androgen Response Element
tggagaacagcctgttctcca

SEQ ID NO: 77 - DNA, 95 bp, Artificial
  MangoII Aptamer + F30 Scaffold
ttgccatgtgtatgtgggtacgaaggagaggagaggaagaggagagtacccacatactctgatgatccttcgggatcattcatggcaatctagga

SEQ ID NO: 78 - DNA, 30 bp, Artificial
  MangoII Aptamer
tacgaaggagaggagaggaagaggagagta

SEQ ID NO: 79 - DNA, 17 bp, Artificial
  Primary Estrogen Response Element
caggtcagcatgacctg

SEQ ID NO: 80 - DNA, 331 bp, Artificial
  ARE/ERE Multiplexed Assay (Single) Nucleic Acid Molecule
taatacgactcactatagactctggaggaatggagaacagcctgttctccattgccatgtgtatgtgggtacgaaggagaggagaggaagaggagagtacccacatactctgatgatccttcgggatcattcatggcaatctaggaaaccccgcggggcctttcgggggtctcgcggggttttttgctctaatacgactcactatagactctggaggaacaggtcagcatgacctgttgccatgtgtatgtgggtacgaaggagaggagaggaagaggagagtacccacatactctgatgatccttcgggatcattcatggcaatctagga